European Patent Specification EP 3 521 456 B1, published January 4, 2023. Title: METHODS AND MEANS FOR ENHANCING RNA PRODUCTION. Applicant: CureVac AG. The sequence listing filed with the application follows.

SEQUENCE LISTING (6 sequences)

SEQ ID NO: 1 - RNA, 589 nt, Artificial Sequence
  G/C optimized mRNA sequence of R1871 coding for Homo sapiens prostate stem cell antigen (HsPSCA)
gggagaaagcuuaccaugaaggccgugcugcucgcgcugcugauggccggccuggcccugcagccggggaccgcccugcugugcuacagcugcaaggcccaggucucgaacgaggacugccugcagguggagaacugcacgcagcugggcgagcagugcuggaccgcccggauccgcgccgugggccugcucaccgugaucagcaagggcugcagccugaacugcguggacgacagccaggacuacuacgugggcaagaagaacaucaccugcugcgacaccgaccugugcaacgccagcggcgcccacgcccugcagcccgcggccgccauccuggcccugcugcccgcccugggccugcugcucuggggccccggccagcugugaccacuaguuauaagacugacuagcccgaugggccucccaacgggcccuccuccccuccuugcaccgagauuaauaaaaaaaaaaaaaaaaaaaaaaaaaaaaaaaaaaaaaaaaaaaaaaaaaaaaaaaaaaaaaaaaugcaucccccccccccccccccccccccccccccccaaaggcucuuuucagagccaccagaauu

SEQ ID NO: 2 - RNA, 1870 nt, Artificial Sequence
  G/C optimized mRNA sequence of R2988 coding for Photinus pyralis luciferase (PpLuc)
gggagaaagcuuaccauggaggacgccaagaacaucaagaagggcccggcgcccuucuacccgcuggaggacgggaccgccggcgagcagcuccacaaggccaugaagcgguacgcccuggugccgggcacgaucgccuucaccgacgcccacaucgaggucgacaucaccuacgcggaguacuucgagaugagcgugcgccuggccgaggccaugaagcgguacggccugaacaccaaccaccggaucguggugugcucggagaacagccugcaguucuucaugccggugcugggcgcccucuucaucggcguggccgucgccccggcgaacgacaucuacaacgagcgggagcugcugaacagcauggggaucagccagccgaccgugguguucgugagcaagaagggccugcagaagauccugaacgugcagaagaagcugcccaucauccagaagaucaucaucauggacagcaagaccgacuaccagggcuuccagucgauguacacguucgugaccagccaccucccgccgggcuucaacgaguacgacuucgucccggagagcuucgaccgggacaagaccaucgcccugaucaugaacagcagcggcagcaccggccugccgaaggggguggcccugccgcaccggaccgccugcgugcgcuucucgcacgcccgggaccccaucuucggcaaccagaucaucccggacaccgccauccugagcguggugccguuccaccacggcuucggcauguucacgacccugggcuaccucaucugcggcuuccgggugguccugauguaccgguucgaggaggagcuguuccugcggagccugcaggacuacaagauccagagcgcgcugcucgugccgacccuguucagcuucuucgccaagagcacccugaucgacaaguacgaccugucgaaccugcacgagaucgccagcgggggcgccccgcugagcaaggaggugggcgaggccguggccaagcgguuccaccucccgggcauccgccagggcuacggccugaccgagaccacgagcgcgauccugaucacccccgagggggacgacaagccgggcgccgugggcaagguggucccguucuucgaggccaaggugguggaccuggacaccggcaagacccugggcgugaaccagcggggcgagcugugcgugcgggggccgaugaucaugagcggcuacgugaacaacccggaggccaccaacgcccucaucgacaaggacggcuggcugcacagcggcgacaucgccuacugggacgaggacgagcacuucuucaucgucgaccggcugaagucgcugaucaaguacaagggcuaccagguggcgccggccgagcuggagagcauccugcuccagcaccccaacaucuucgacgccggcguggccgggcugccggacgacgacgccggcgagcugccggccgcggugguggugcuggagcacggcaagaccaugacggagaaggagaucgucgacuacguggccagccaggugaccaccgccaagaagcugcggggcggcgugguguucguggacgaggucccgaagggccugaccgggaagcucgacgcccggaagauccgcgagauccugaucaaggccaagaagggcggcaagaucgccgugugaggacuaguuauaagacugacuagcccgaugggccucccaacgggcccuccuccccuccuugcaccgagauuaauaaaaaaaaaaaaaaaaaaaaaaaaaaaaaaaaaaaaaaaaaaaaaaaaaaaaaaaaaaaaaaaaugcaucccccccccccccccccccccccccccccccaaaggcucuuuucagagccaccagaauu

SEQ ID NO: 3 - RNA, 5337 nt, Artificial Sequence
  G/C optimized mRNA sequence of R1626 coding for Homo sapiens Mucin-1 signal peptide/epidermal growth factor receptor/Mucin-1 fusion protein (EGFR/Mucin-1)
gggagaaagcuuaccaugacccccggcacccagagcccguucuuccugcuccugcugcucacggugcugaccgucgugaccgggaugcggccgagcggcaccgccggggcggcccugcucgcccugcuggccgcccugugccccgccucgcgcgcgcuggaggagaagaaggugugccagggcacgagcaacaagcugacccagcucggcaccuucgaggaccacuuccugagccugcagcggauguucaacaacugcgaggucgugcugggcaaccuggagaucaccuacgugcagcggaacuacgaccugagcuuccucaagaccauccaggagguggccggcuacgugcugaucgcccugaacaccguggagcggaucccgcuggagaaccugcagaucauccggggcaacauguacuacgagaacagcuacgcccuggccguccucagcaacuacgacgccaacaagacggggcugaaggagcugccgaugcggaaccugcaggagauccugcacggcgcggugcgcuucucgaacaacccggcccugugcaacguggagagcauccaguggcgggacaucgugagcagcgacuuccucagcaacaugagcauggacuuccagaaccaccugggcucgugccagaagugcgacccgagcugcccgaacggcagcugcuggggcgccggcgaggagaacugccagaagcugaccaagaucaucugcgcccagcagugcagcgggcggugccggggcaagagccccagcgacugcugccacaaccagugcgccgccggcugcaccggcccgcgggagucggacugccuggugugccggaaguuccgcgacgaggcgaccugcaaggacaccugcccgccgcugaugcuguacaacccgaccacguaccagauggacgugaacccggagggcaaguacagcuucggcgccaccugcgucaagaagugcccccggaacuacguggugaccgaccacgggagcugcgugcgggccugcggcgccgacagcuacgagauggaggaggacggcgugcggaagugcaagaagugcgagggcccgugccggaaggugugcaacggcaucggcaucggggaguucaaggacagccucagcaucaacgccaccaacaucaagcacuucaagaacugcaccucgaucagcggcgaccugcacauccugccggucgccuuccggggcgacagcuucacccacacgccgccgcuggacccgcaggagcuggacauccugaagaccgugaaggagaucaccggcuuccuccugauccaggcguggcccgagaaccgcaccgaccugcacgccuucgagaaccuggagaucauccggggccggaccaagcagcacggccaguucagccuggccguggugagccugaacaucaccagccucgggcugcggucgcugaaggagaucagcgacggcgacgugaucaucagcggcaacaagaaccugugcuacgccaacacgaucaacuggaagaagcuguucggcaccagcggccagaagaccaagaucaucagcaaccggggcgagaacagcugcaaggccaccgggcaggugugccacgcccugugcucgccggagggcugcuggggcccggagccgcgggacugcgucagcugccgcaacgugagccggggccgggagugcguggacaagugcaaccuccuggagggcgagccgcgggaguucguggagaacagcgagugcauccagugccacccggagugccugccccaggcgaugaacaucaccugcaccggccgggggccggacaacugcauccagugcgcccacuacaucgacggcccgcacugcgugaagacgugcccggccggcgugaugggcgagaacaacacccuggucuggaaguacgccgacgccggccacgugugccaccugugccacccgaacugcaccuacggcugcaccgggccgggccuggagggcugccccaccaacggcccgaagaucccgagcaucgccaccggcauggugggcgcgcuccugcugcugcuggugguggcccuggggaucggccucuucaugcggcgccggcacaucgugcggaagcggacgcugcggcggcugcugcaggagcgcgagcuggucgagccgcugaccccgagcggcgaggccccgaaccaggcccuccugcggauccugaaggagaccgaguucaagaagaucaaggugcugggcucgggcgccuucggcaccguguacaaggggcuguggauccccgagggcgagaaggugaagaucccgguggccaucaaggagcugcgggaggcgaccagcccgaaggccaacaaggagauccucgacgaggccuacgugauggccagcgucgacaacccgcacgugugccggcugcugggcaucugccugaccagcacggugcagcugaucacccagcugaugccguucggcugccuccuggacuacgugcgggagcacaaggacaacaucggcagccaguaccugcugaacuggugcgugcagaucgccaagggcaugaacuaccuggaggaccggcgccuggugcaccgggaccucgccgcgcggaacguccuggugaagaccccgcagcacgugaagaucaccgacuucgggcuggccaagcugcugggcgccgaggagaaggaguaccacgccgagggcggcaaggugcccaucaaguggauggcccuggagagcauccuccaccggaucuacacccaccagucggacguguggagcuacggcgugaccgucugggagcugaugacguucggcagcaagccguacgacgggaucccggccagcgagaucagcagcauccuggagaagggcgagcggcugccgcagccgccgaucugcaccaucgacguguacaugaucauggugaagugcuggaugaucgacgcggacucgcggcccaaguuccgcgagcugaucaucgaguucagcaagauggcccgggacccgcagcgguaccuggugauccagggcgacgagcggaugcaccucccgagcccgaccgacagcaacuucuaccgggcccugauggacgaggaggacauggacgacgugguggacgccgacgaguaccugaucccgcagcagggcuucuucagcagcccgucgaccagccggaccccgcugcugagcagccugagcgccaccagcaacaacucgacggucgccugcaucgaccgcaacggccuccagagcugccccaucaaggaggacagcuuccugcagcgguacagcagcgacccgaccggcgcgcugaccgaggacagcaucgacgacaccuuccugccggugccggaguacaucaaccagucggugccgaagcggcccgccgggagcgugcagaacccgguguaccacaaccagccgcugaacccggccccgagccgggacccgcacuaccaggacccccacagcaccgccgugggcaacccggaguaccugaacaccguccagccgacgugcgugaacagcaccuucgacagcccggcccacugggcccagaagggcucgcaccagaucagccucgacaacccggacuaccagcaggacuucuucccgaaggaggcgaagcccaacggcaucuucaagggcagcaccgccgagaacgccgaguaccugcggguggccccgcagagcagcgaguucaucggcgccuccggccacgccagcuccacccccgggggcgagaaggagacgagcgccacccagcgguccagcgugcccuccagcaccgagaagaacgcggucuccaugaccagcuccgugcugagcucccacagccccggguccggcagcuccacgacccagggccaggacgugacccucgccccggccaccgagcccgccagcggguccgccgcgacguggggccaggacgucaccagcgugcccgugacccgccccgcccuggggagcaccacgccgcccgcccacgacgucaccuccgcccccgacaacaagcccgcgccgggcagcaccgccccccccgcccacggggugaccuccgcccccgacacgcggccggcccccggcagcaccgcgccccccgcccacggcgugaccuccgccccggacacccgcccggcccccggcagcaccgccccccccgcccacggggugaccuccgccccggacacgcggcccgcccccggcagcaccgccccgcccgcccacggcgucacguccgcgcccgacaaccgccccgcccuggggagcaccgccccgcccgugcacaacgugaccuccgccagcggcuccgcgagcggguccgccagcacccucguccacaacggcacguccgcccgggccaccaccacccccgccagcaaguccacgcccuucagcaucccgucccaccacagcgacacccccaccacccuggcgucccacagcacgaagaccgacgccuccagcacccaccacuccagcgugcccccgcugaccagcuccaaccacagcacguccccgcagcucagcaccgggguguccuucuucuuccugagcuuccacaucuccaaccugcaguucaacagcucccucgaggaccccagcaccgacuacuaccaggagcugcagcgggacaucuccgagauguuccugcagaucuacaagcagggcggcuuccucgggcugagcaacaucaaguuccgccccggcuccgucguggugcagcugacccucgccuuccgggaggggacgaucaacguccacgacguggagacccaguucaaccaguacaagaccgaggccgccagccgcuacaaccugaccaucuccgacgugagcgucuccgacgugcccuucccguucagcgcgcaguccggcgccggcgugcccggggccgugugccagugccggcgcaagaacuacgggcagcucgacaucuuccccgcccgggacacguaccacccgaugagcgaguacccgaccuaccacacccacggccgcuacgucccccccagcuccaccgaccggagccccuacgagaagguguccgccgggaacggcggcagcucccugagcuacaccaacccggcgguggccgccgccuccgccaaccuggaggaccagguggacccccggcugaucgacggcaagugaggacuaguuauaagacugacuagcccgaugggccucccaacgggcccuccuccccuccuugcaccgagauuaauaaaaaaaaaaaaaaaaaaaaaaaaaaaaaaaaaaaaaaaaaaaaaaaaaaaaaaaaaaaaaaaauauuccccccccccccccccccccccccccccccucuag

SEQ ID NO: 4 - RNA, 547 nt, Artificial Sequence
  Non-coding immunostimulatory RNA sequence of R2025
gggagaaagcucaagcuuauccaaguaggcuggucaccuguacaacguagccgguauuuuuuuuuuuuuuuuuuuuuugaccgucucaagguccaaguuagucugccuauaaaggugcggauccacagcugaugaaagacuugugcgguacgguuaaucuccccuuuuuuuuuuuuuuuuuuuuuaguaaaugcgucuacugaauccagcgaugaugcuggcccagaucuucgaccacaagugcauauaguagucaucgagggucgccuuuuuuuuuuuuuuuuuuuuuuuggcccaguucugagacuucgcuagagacuacaguuacagcugcaguaguaaccacugcggcuauugcaggaaaucccguucagguuuuuuuuuuuuuuuuuuuuuccgcucacuaugauuaagaaccagguggagugucacugcucucgaggucucacgagagcgcucgauacaguccuuggaagaaucuuuuuuuuuuuuuuuuuuuuuugugcgacgaucacagagaacuucuauucaugcaggucugcucuag

SEQ ID NO: 5 - RNA, 52 nt, Artificial Sequence
  hammerhead ribozyme HHNUH2d
gcauggcugaugaggccucgaccgauaggucgaggccgaaaagcuuucuccc

SEQ ID NO: 6 - RNA, 2083 nt, Artificial Sequence
  G/C optimized mRNA sequence encoding HA from Influenza A H1N1 (Netherlands 2009)
ggggcgcugccuacggagguggcagccaucuccuucucggcaucaagcuuaccaugaaggccauccuggugguccuccuguacaccuucgccaccgcgaacgccgacacgcugugcaucggcuaccacgccaacaacagcaccgacaccguggacaccgugcucgagaagaacgucacggugacccacuccgugaaccugcuggaggacaagcacaacgggaagcucugcaagcugcggggcgucgccccgcugcaccucgggaagugcaacaucgccggcuggauccuggggaacccggagugcgagagccuguccaccgcgagcuccuggagcuacaucguggagaccuccagcuccgacaacggcacgugcuaccccggcgacuucaucgacuacgaggagcuccgcgagcagcugagcuccgugagcuccuucgagcgguucgagaucuuccccaagaccagcuccuggcccaaccacgacagcaacaagggggucaccgccgccugcccgcacgccggcgcgaaguccuucuacaagaaccugaucuggcucgugaagaaggggaacagcuaccccaagcuguccaagagcuacaucaacgacaagggcaaggaggugcugguccucugggggauccaccaccccagcaccuccgccgaccagcagagccuguaccagaacgccgacgccuacguguucgugggcuccagccgcuacuccaagaaguucaagcccgagaucgccauccggccgaagguccgcgaccaggagggccggaugaacuacuacuggacgcugguggagcccggggacaagaucaccuucgaggcgaccggcaaccucguggucccccgcuacgccuucgccauggagcggaacgccgggagcggcaucaucaucuccgacacccccgugcacgacugcaacacgaccugccagaccccgaagggcgccaucaacaccagccugcccuuccagaacauccaccccaucacgaucgggaagugccccaaguacgugaaguccaccaagcugcgccucgcgaccggccugcggaacgucccgagcauccagucccgcgggcuguucggcgccaucgccggguucaucgagggcggcuggaccgggaugguggacggcugguacggguaccaccaccagaacgagcagggcagcggguacgccgccgaccucaaguccacgcagaacgcgaucgacgagaucaccaacaaggugaacagcgucaucgagaagaugaacacccaguucaccgccgugggcaaggaguucaaccaccuggagaagcggaucgagaaccugaacaagaaggucgacgacggcuuccucgacaucuggacguacaacgccgagcugcuggugcuccuggagaacgagcgcacccuggacuaccacgacuccaacgugaagaaccucuacgagaagguccggagccagcugaagaacaacgccaaggagaucgggaacggcugcuucgaguucuaccacaagugcgacaacaccugcauggaguccgugaagaacgggaccuacgacuaccccaaguacagcgaggaggccaagcugaaccgcgaggagaucgacggcgugaagcucgaguccacgcggaucuaccagauccuggcgaucuacagcaccgucgccagcucccuggugcucguggucagccugggggccaucuccuucuggaugugcagcaacggcucccugcagugccgcaucugcaucugaccacuagugcaucacauuuaaaagcaucucagccuaccaugagaauaagagaaagaaaaugaagaucaauagcuuauucaucucuuuuucuuuuucguugguguaaagccaacacccugucuaaaaaacauaaauuucuuuaaucauuuugccucuuuucucugugcuucaauuaauaaaaaauggaaagaaccuagaucuaaaaaaaaaaaaaaaaaaaaaaaaaaaaaaaaaaaaaaaaaaaaaaaaaaaaaaaaaaaaaaaaugcaucccccccccccccccccccccccccccccccaaaggcucuuuucagagccaccagaauu